European Patent Specification EP 3 256 156 B1, published February 12, 2025. Title: Immunotherapeutic vaccine and antibody combination therapy. Applicant: TRANSGENE SA. The sequence listing filed with the application follows.

SEQUENCE LISTING (6 sequences)

SEQ ID NO: 1 - protein, 557 aa, Homo sapiens
MTPGTQSPFFLLLLLTVLTVVTGSGHASSTPGGEKETSATQRSSVPSSTEKNAVSMTSSVLSSHSPGSGSSTTQGQDVTLAPATEPASGSAATWGQDVTSVPVTRPALGSTTPPAHDVTSAPDNKPAPSPGSTAPPAHGVTSAPDTRPAPGSTAPPAHGVTSAPDTRPAPGSTAPPAHGVTSAPDTRPAPGSTAPPAHGVTSAPDTRPAPGSTAPPGHGVTSAPDTRPAPGSTAPPAHGVTSAPDNRPALGSTAPPVHNVTSASGSASGSASTLVHNGTSARATTTPASKSTPFSIPSHHSDTPTTLASHSTKTDASSTHHSTVPPLTSSNHSTSPQLSTGVSFFFLSFHISNLQFNSSLEDPSTDYYQELQRDISEMFLQIYKQGGFLGLSNIKFRPGSVVVQLTLAFREGTINVHDVETQFNQYKTEAASRYNLTISDVSVSDVPFPFSAQSGAGVPGWGIALLVLVCVLVALAIVYLIALAVCQCRRKNYGQLDIFPARDTYHPMSEYPTYHTHGRYVPPSSTDRSPYEKVSAGNGGSSLSYTNPAVAATSANL

SEQ ID NO: 2 - DNA, 1674 bp, Homo sapiens
atgacaccgggcacccagtctcctttcttcctgctgctgctcctcacagtgcttacagttgttacaggttctggtcatgcaagctctaccccaggtggagaaaaggagacttcggctacccagagaagttcagtgcccagctctactgagaagaatgctgtgagtatgaccagcagcgtactctccagccacagccccggttcaggctcctccaccactcagggacaggatgtcactctggccccggccacggaaccagcttcaggttcagctgccacctggggacaggatgtcacctcggtcccagtcaccaggccagccctgggctccaccaccccgccagcccacgatgtcacctcagccccggacaacaagccagccccatctccaggctccaccgcccccccagcccacggtgtcacctcggccccggacaccaggccggcaccaggaagcacagcaccacccgcgcatggtgtaacatctgcccctgatacacgtcctgctcccggtagtactgcgccgcctgcacacggggtgacgtctgctcccgacactcggccggcgcctgggtcaacggctcctccggcacatggagttacttctgcgccagacacgcgacccgctccaggtagtacggcgccaccggggcatggagtgacatctgcgcccgatactaggccggccccgggctccaccgcccccccagcccatggtgtcacctcggccccggacaacaggcccgccttgggctccaccgcccctccagtccacaatgtcacctcggcctcaggctctgcatcaggctcagcttctactctggtgcacaacggcacctctgccagggctaccacaaccccagccagcaagagcactccattctcaattcccagccaccactctgatactcctaccacccttgccagccatagcaccaagactgatgccagtagcactcaccatagcacggtacctcctctcacctcctccaatcacagcacttctccccagttgtctactggggtctctttctttttcctgtcttttcacatttcaaacctccagtttaattcctctctggaagatcccagcaccgactactaccaagagctgcagagagacatttctgaaatgtttttgcagatttataaacaagggggttttctgggcctctccaatattaagttcaggccaggatctgtggtggtacaattgactctggccttccgagaaggtaccatcaatgtccacgacgtggagacacagttcaatcagtataaaacggaagcagcctctcgatataacctgacgatctcagacgtcagcgtgagtgatgtgccatttcctttctctgcccagtctggggctggggtgccaggctggggcatcgcgctgctggtgctggtctgtgttctggttgcgctggccattgtctatctcattgccttggctgtctgtcagtgccgccgaaagaactacgggcagctggacatctttccagcccgggatacctaccatcctatgagcgagtaccccacctaccacacccatgggcgctatgtgccccctagcagtaccgatcgtagcccctatgagaaggtttctgcaggtaatggtggcagcagcctctcttacacaaacccagcagtggcagccacttctgccaacttgtag

SEQ ID NO: 3 - protein, 1047 aa, Escherichia coli
MSFTLTNKNVIFVAGLGGIGLDTSKELLKRDPVVLQRRDWENPGVTQLNRLAAHPPFASWRNSEEARTDRPSQQLRSLNGEWRFAWFPAPEAVPESWLECDLPEADTVVVPSNWQMHGYDAPIYTNVTYPITVNPPFVPTENPTGCYSLTFNVDESWLQEGQTRIIFDGVNSAFHLWCNGRWVGYGQDSRLPSEFDLSAFLRAGENRLAVMVLRWSDGSYLEDQDMWRMSGIFRDVSLLHKPTTQISDFHVATRFNDDFSRAVLEAEVQMCGELRDYLRVTVSLWQGETQVASGTAPFGGEIIDERGGYADRVTLRLNVENPKLWSAEIPNLYRAVVELHTADGTLIEAEACDVGFREVRIENGLLLLNGKPLLIRGVNRHEHHPLHGQVMDEQTMVQDILLMKQNNFNAVRCSHYPNHPLWYTLCDRYGLYVVDEANIETHGMVPMNRLTDDPRWLPAMSERVTRMVQRDRNHPSVIIWSLGNESGHGANHDALYRWIKSVDPSRPVQYEGGGADTTATDIICPMYARVDEDQPFPAVPKWSIKKWLSLPGETRPLILCEYAHAMGNSLGGFAKYWQAFRQYPRLQGGFVWDWVDQSLIKYDENGNPWSAYGGDFGDTPNDRQFCMNGLVFADRTPHPALTEAKHQQQFFQFRLSGQTIEVTSEYLFRHSDNELLHWMVALDGKPLASGEVPLDVAPQGKQLIELPELPQPESAGQLWLTVRVVQPNATAWSEAGHISAWQQWRLAENLSVTLPAASHAIPHLTTSEMDFCIELGNKRWQFNRQSGFLSQMWIGDKKQLLTPLRDQFTRAPLDNDIGVSEATRIDPNAWVERWKAAGHYQAEAALLQCTADTLADAVLITTAHAWQHQGKTLFISRKTYRIDGSGQMAITVDVEVASDTPHPARIGLNCQLAQVAERVNWLGLGPQENYPDRLTAACFDRWDLPLSDMYTPYVFPSENGLRCGTRELNYGPHQWRGDFQFNISRYSQQQLMETSHRHLLHAEEGTWLNIDGFHMGIGGDDSWSPSVSAELQLSAGRYHYQLVWCQK

SEQ ID NO: 4 - DNA, 114 bp, Vaccinia virus
tttattctatacttaaaaaatgaaaataaatacaaaggttcttgagggttgtgttaaattgaaagcgagaaataatcataaattatttcattatcgcgatatccgttaagtttg

SEQ ID NO: 5 - DNA, 46 bp, artificial sequence
  PCR primer for LacZ cloning
ccaccttaattaagccgccaccatgtcgtttactttgaccaacaag

SEQ ID NO: 6 - DNA, 43 bp, artificial sequence
  PCR primer for LacZ cloning
accaactcgagagaaaaattatttttgacaccagaccaactgg